European Patent Application EP 4 324 484 A1, published February 21, 2024. Title: Catalyst augmented target specific polypeptide. Applicant: Technische Universiaet Berlin. Application EP. The sequence listing filed with the application follows.

SEQUENCE LISTING (4 sequences)

SEQ ID NO: 1 - protein, 5 aa, synthetic construct
HRGDH

SEQ ID NO: 2 - protein, 5 aa, synthetic construct
GGGGS

SEQ ID NO: 3 - protein, 12 aa, synthetic construct
ENLYQSHHHHHH

SEQ ID NO: 4 - protein, 138 aa, synthetic construct
QVQLQESGGGSVQAGGSLKLTCAASGYIFNSCGMGWYRQSPGRERELVSRISGDGDTWHKESVKGRFTISQDNVKKTLYLQMNSLKPEDTAVYFCAVCYNLETYWGQGTQVTVSSGGGGSHRGDHENLYFQSHHHHHH